European Patent Specification EP 3 630 787 B1, published January 15, 2025. Title: Tetramolecular parallel G-quadruplex-forming hydrophobically modified oligonucleotides. Applicant: INSERM CNRS Université de Bordeaux. The sequence listing filed with the application follows.

SEQUENCE LISTING (2 sequences)

SEQ ID NO: 1 - DNA, 19 bp, Artificial Sequence
  sequence of modified "G4 prone" oligonucleotide
ttagttggggttcagttgg

SEQ ID NO: 2 - DNA, 19 bp, Artificial Sequence
  sequence of "scramble" oligonucleotide
tgtagtaggttgtgtctgg